European Patent Specification EP 3 704 244 B1, published August 14, 2024. Title: Vector Construct. Applicant: Nextera AS. The sequence listing filed with the application follows.

SEQUENCE LISTING (61 sequences)

SEQ ID NO: 1 - DNA, 114 bp, Artificial Sequence
  Artificial Sequence
atgaacaataacgatctctttcagacatcacgtcagcgttttttggcacaactcggcggcttaaccgtcgccgggatgctggggccgtcattgttaacgccgcgacgtgcgact

SEQ ID NO: 2 - protein, 38 aa, Artificial Sequence
  Artificial Sequence
MNNNDLFQTSRQRFLAQLGGLTVAGMLGPSLLTPRRAT

SEQ ID NO: 3 - DNA, 705 bp, Artificial Sequence
  Artificial Sequence
gtttctaaaggtgaagaagacaacatggcttctctgccggctacccacgaactgcacatcttcggttctatcaacggtgttgacttcgacatggttggtcagggtaccggtaacccgaacgacggttacgaagaactgaacctgaaatctaccaaaggtgacctgcagttctctccgtggatcttagttccgcacatcggttacggtttccaccagtacctgccgtacccggacggtatgtctccgttccaggctgctatggttgacggttctggttaccaggttcaccgtaccatgcagttcgaagacggtgcttctctgaccgttaactaccgttacacctacgaaggttctcacatcaaaggtgaagctcaggttaaaggtaccggtttcccggctgacggtccggttatgaccaactctctgaccgctgctgactggtgccgttctaaaaaaacctacccgaacgacaaaaccatcatctctaccttcaaatggtcttacaccaccggtaacggtaaacgttaccgttctaccgctcgtaccacctacaccttcgctaaaccgatggctgctaactacctgaaaaaccagccgatgtacgttttccgtaaaaccgaactgaaacactctaaaaccgaactgaacttcaaagaatggcagaaagctttcaccgacgttatgggtatggacgaactgtacaaa

SEQ ID NO: 4 - protein, 235 aa, Artificial Sequence
  Artificial Sequence
VSKGEEDNMASLPATHELHIFGSINGVDFDMVGQGTGNPNDGYEELNLKSTKGDLQFSPWILVPHIGYGFHQYLPYPDGMSPFQAAMVDGSGYQVHRTMQFEDGASLTVNYRYTYEGSHIKGEAQVKGTGFPADGPVMTNSLTAADWCRSKKTYPNDKTIISTFKWSYTTGNGKRYRSTARTTYTFAKPMAANYLKNQPMYVFRKTELKHSKTELNFKEWQKAFTDVMGMDELYK

SEQ ID NO: 5 - DNA, 24 bp, Artificial Sequence
  Artificial Sequence
ggcggtggcagcggcggtggcagc

SEQ ID NO: 6 - protein, 8 aa, Artificial Sequence
  Artificial Sequence
GGGSGGGS

SEQ ID NO: 7 - DNA, 150 bp, Artificial Sequence
  Artificial Sequence
gctgagggtgacgatcccgcaaaagcggcctttaactccctgcaagcctcagcgaccgaatatatcggttatgcgtgggcgatggttgttgtcattgtcggcgcaactatcggtatcaagctgtttaagaaattcacctcgaaagcaagc

SEQ ID NO: 8 - protein, 50 aa, Artificial Sequence
  Artificial Sequence
AEGDDPAKAAFNSLQASATEYIGYAWAMVVVIVGATIGIKLFKKFTSKAS

SEQ ID NO: 9 - DNA, 24 bp, Artificial Sequence
  Artificial Sequence
gattacaaggatgacgatgacaag

SEQ ID NO: 10 - protein, 8 aa, Artificial Sequence
  Artificial Sequence
DYKDDDDK

SEQ ID NO: 11 - DNA, 1221 bp, Artificial Sequence
  Artificial Sequence
gctgaaactgttgaaagttgtttagcaaaaccccatacagaaaattcatttactaacgtctggaaagacgacaaaactttagatcgttacgctaactatgagggctgtctgtggaatgctacaggcgttgtagtttgtactggtgacgaaactcagtgttacggtacatgggttcctattgggcttgctatccctgaaaatgagggtggtggctctgagggtggcggttctgagggtggcggttctgagggtggcggtactaaacctcctgagtacggtgatacacctattccgggctatacttatatcaaccctctcgacggcacttatccgcctggtactgagcaaaaccccgctaatcctaatccttctcttgaggagtctcagcctcttaatactttcatgtttcagaataataggttccgaaataggcagggggcattaactgtttatacgggcactgttactcaaggcactgaccccgttaaaacttattaccagtacactcctgtatcatcaaaagccatgtatgacgcttactggaacggtaaattcagagactgcgctttccattctggctttaatgaggatccattcgtttgtgaatatcaaggccaatcgtctgacctgcctcaacctcctgtcaatgctggcggcggctctggtggtggttctggtggcggctctgagggtggtggctctgagggtggcggttctgagggtggcggctctgagggaggcggttccggtggtggctctggttccggtgattttgattatgaaaagatggcaaacgctaataagggggctatgaccgaaaatgccgatgaaaacgcgctacagtctgacgctaaaggcaaacttgattctgtcgctactgattacggtgctgctatcgatggtttcattggtgacgtttccggccttgctaatggtaatggtgctactggtgattttgctggctctaattcccaaatggctcaagtcggtgacggtgataattcacctttaatgaataatttccgtcaatatttaccttccctccctcaatcggttgaatgtcgcccttttgtctttggcgctggtaaaccatatgaattttctattgattgtgacaaaataaacttattccgtggtgtctttgcgtttcttttatatgttgccacctttatgtatgtattttctacgtttgctaacatactgcgtaataaggagtcttaa

SEQ ID NO: 12 - protein, 406 aa, Artificial Sequence
  Artificial Sequence
AETVESCLAKPHTENSFTNVWKDDKTLDRYANYEGCLWNATGVVVCTGDETQCYGTWVPIGLAIPENEGGGSEGGGSEGGGSEGGGTKPPEYGDTPIPGYTYINPLDGTYPPGTEQNPANPNPSLEESQPLNTFMFQNNRFRNRQGALTVYTGTVTQGTDPVKTYYQYTPVSSKAMYDAYWNGKFRDCAFHSGFNEDPFVCEYQGQSSDLPQPPVNAGGGSGGGSGGGSEGGGSEGGGSEGGGSEGGGSGGGSGSGDFDYEKMANANKGAMTENADENALQSDAKGKLDSVATDYGAAIDGFIGDVSGLANGNGATGDFAGSNSQMAQVGDGDNSPLMNNFRQYLPSLPQSVECRPFVFGAGKPYEFSIDCDKINLFRGVFAFLLYVATFMYVFSTFANILRNKES

SEQ ID NO: 13 - protein, 112 aa, Artificial Sequence
  Artificial Sequence
MPVLLGIPLLLRFLGFLLVTLFGYLLTFLKKGFGKIAIAISLFLALIIGLNSILVGYLSDISAQLPSDFVQGVQLILPSNALPCFYVILSVKAAIFIFDVKQKIVSYLDWDK

SEQ ID NO: 14 - protein, 33 aa, Artificial Sequence
  Artificial Sequence
MEQVADFDTIYQAMIQISVVLCFALGIIAGGQR

SEQ ID NO: 15 - protein, 32 aa, Artificial Sequence
  Artificial Sequence
MSVLVYSFASFVLGWCLRSGITYFTRLMETSS

SEQ ID NO: 16 - protein, 273 aa, Artificial Sequence
  Artificial Sequence
VSKGEEDNMASLPATHELHIFGSINGVDFDMVGQGTGNPNDGYEELNLKSTKGDLQFSPWILVPHIGYGFHQYLPYPDGMSPFQAAMVDGSGYQVHRTMQFEDGASLTVNYRYTYEGSHIKGEAQVKGTGFPADGPVMTNSLTAADWCRSKKTYPNDKTIISTFKWSYTTGNGKRYRSTARTTYTFAKPMAANYLKNQPMYVFRKTELKHSKTELNFKEWQKAFTDVMGMDELYKGGGSGGGSAEGDDPAKAAFNSLQASATEYIGYAWAMVV

SEQ ID NO: 17 - DNA, 819 bp, Artificial Sequence
  Artificial Sequence
gtttctaaaggtgaagaagacaacatggcttctctgccggctacccacgaactgcacatcttcggttctatcaacggtgttgacttcgacatggttggtcagggtaccggtaacccgaacgacggttacgaagaactgaacctgaaatctaccaaaggtgacctgcagttctctccgtggatcttagttccgcacatcggttacggtttccaccagtacctgccgtacccggacggtatgtctccgttccaggctgctatggttgacggttctggttaccaggttcaccgtaccatgcagttcgaagacggtgcttctctgaccgttaactaccgttacacctacgaaggttctcacatcaaaggtgaagctcaggttaaaggtaccggtttcccggctgacggtccggttatgaccaactctctgaccgctgctgactggtgccgttctaaaaaaacctacccgaacgacaaaaccatcatctctaccttcaaatggtcttacaccaccggtaacggtaaacgttaccgttctaccgctcgtaccacctacaccttcgctaaaccgatggctgctaactacctgaaaaaccagccgatgtacgttttccgtaaaaccgaactgaaacactctaaaaccgaactgaacttcaaagaatggcagaaagctttcaccgacgttatgggtatggacgaactgtacaaaggcggtggcagcggcggtggcagcgctgagggtgacgatcccgcaaaagcggcctttaactccctgcaagcctcagcgaccgaatatatcggttatgcgtgggcgatggttgtt

SEQ ID NO: 18 - protein, 293 aa, Artificial Sequence
  Artificial Sequence
VSKGEEDNMASLPATHELHIFGSINGVDFDMVGQGTGNPNDGYEELNLKSTKGDLQFSPWILVPHIGYGFHQYLPYPDGMSPFQAAMVDGSGYQVHRTMQFEDGASLTVNYRYTYEGSHIKGEAQVKGTGFPADGPVMTNSLTAADWCRSKKTYPNDKTIISTFKWSYTTGNGKRYRSTARTTYTFAKPMAANYLKNQPMYVFRKTELKHSKTELNFKEWQKAFTDVMGMDELYKGGGSGGGSAEGDDPAKAAFNSLQASATEYIGYAWAMVVVIVGATIGIKLFKKFTSKAS

SEQ ID NO: 19 - DNA, 879 bp, Artificial Sequence
  Artificial Sequence
gtttctaaaggtgaagaagacaacatggcttctctgccggctacccacgaactgcacatcttcggttctatcaacggtgttgacttcgacatggttggtcagggtaccggtaacccgaacgacggttacgaagaactgaacctgaaatctaccaaaggtgacctgcagttctctccgtggatcttagttccgcacatcggttacggtttccaccagtacctgccgtacccggacggtatgtctccgttccaggctgctatggttgacggttctggttaccaggttcaccgtaccatgcagttcgaagacggtgcttctctgaccgttaactaccgttacacctacgaaggttctcacatcaaaggtgaagctcaggttaaaggtaccggtttcccggctgacggtccggttatgaccaactctctgaccgctgctgactggtgccgttctaaaaaaacctacccgaacgacaaaaccatcatctctaccttcaaatggtcttacaccaccggtaacggtaaacgttaccgttctaccgctcgtaccacctacaccttcgctaaaccgatggctgctaactacctgaaaaaccagccgatgtacgttttccgtaaaaccgaactgaaacactctaaaaccgaactgaacttcaaagaatggcagaaagctttcaccgacgttatgggtatggacgaactgtacaaaggcggtggcagcggcggtggcagcgctgagggtgacgatcccgcaaaagcggcctttaactccctgcaagcctcagcgaccgaatatatcggttatgcgtgggcgatggttgttgtcattgtcggcgcaactatcggtatcaagctgtttaagaaattcacctcgaaagcaagc

SEQ ID NO: 20 - protein, 334 aa, Artificial Sequence
  Artificial Sequence
MNNNDLFQTSRQRFLAQLGGLTVAGMLGPSLLTPRRATAAGVSKGEEDNMASLPATHELHIFGSINGVDFDMVGQGTGNPNDGYEELNLKSTKGDLQFSPWILVPHIGYGFHQYLPYPDGMSPFQAAMVDGSGYQVHRTMQFEDGASLTVNYRYTYEGSHIKGEAQVKGTGFPADGPVMTNSLTAADWCRSKKTYPNDKTIISTFKWSYTTGNGKRYRSTARTTYTFAKPMAANYLKNQPMYVFRKTELKHSKTELNFKEWQKAFTDVMGMDELYKGGGSGGGSAEGDDPAKAAFNSLQASATEYIGYAWAMVVVIVGATIGIKLFKKFTSKAS

SEQ ID NO: 21 - DNA, 1002 bp, Artificial Sequence
  Artificial Sequence
atgaacaataacgatctctttcagacatcacgtcagcgttttttggcacaactcggcggcttaaccgtcgccgggatgctggggccgtcattgttaacgccgcgacgtgcgactgcggcgggcgtttctaaaggtgaagaagacaacatggcttctctgccggctacccacgaactgcacatcttcggttctatcaacggtgttgacttcgacatggttggtcagggtaccggtaacccgaacgacggttacgaagaactgaacctgaaatctaccaaaggtgacctgcagttctctccgtggatcttagttccgcacatcggttacggtttccaccagtacctgccgtacccggacggtatgtctccgttccaggctgctatggttgacggttctggttaccaggttcaccgtaccatgcagttcgaagacggtgcttctctgaccgttaactaccgttacacctacgaaggttctcacatcaaaggtgaagctcaggttaaaggtaccggtttcccggctgacggtccggttatgaccaactctctgaccgctgctgactggtgccgttctaaaaaaacctacccgaacgacaaaaccatcatctctaccttcaaatggtcttacaccaccggtaacggtaaacgttaccgttctaccgctcgtaccacctacaccttcgctaaaccgatggctgctaactacctgaaaaaccagccgatgtacgttttccgtaaaaccgaactgaaacactctaaaaccgaactgaacttcaaagaatggcagaaagctttcaccgacgttatgggtatggacgaactgtacaaaggcggtggcagcggcggtggcagcgctgagggtgacgatcccgcaaaagcggcctttaactccctgcaagcctcagcgaccgaatatatcggttatgcgtgggcgatggttgttgtcattgtcggcgcaactatcggtatcaagctgtttaagaaattcacctcgaaagcaagc

SEQ ID NO: 22 - protein, 342 aa, Artificial Sequence
  Artificial Sequence
MNNNDLFQTSRQRFLAQLGGLTVAGMLGPSLLTPRRATAADYKDDDDKGVSKGEEDNMASLPATHELHIFGSINGVDFDMVGQGTGNPNDGYEELNLKSTKGDLQFSPWILVPHIGYGFHQYLPYPDGMSPFQAAMVDGSGYQVHRTMQFEDGASLTVNYRYTYEGSHIKGEAQVKGTGFPADGPVMTNSLTAADWCRSKKTYPNDKTIISTFKWSYTTGNGKRYRSTARTTYTFAKPMAANYLKNQPMYVFRKTELKHSKTELNFKEWQKAFTDVMGMDELYKGGGSGGGSAEGDDPAKAAFNSLQASATEYIGYAWAMVVVIVGATIGIKLFKKFTSKAS

SEQ ID NO: 23 - DNA, 1026 bp, Artificial Sequence
  Artificial Sequence
atgaacaataacgatctctttcagacatcacgtcagcgttttttggcacaactcggcggcttaaccgtcgccgggatgctggggccgtcattgttaacgccgcgacgtgcgactgcggcggattacaaggatgacgatgacaagggcgtttctaaaggtgaagaagacaacatggcttctctgccggctacccacgaactgcacatcttcggttctatcaacggtgttgacttcgacatggttggtcagggtaccggtaacccgaacgacggttacgaagaactgaacctgaaatctaccaaaggtgacctgcagttctctccgtggatcttagttccgcacatcggttacggtttccaccagtacctgccgtacccggacggtatgtctccgttccaggctgctatggttgacggttctggttaccaggttcaccgtaccatgcagttcgaagacggtgcttctctgaccgttaactaccgttacacctacgaaggttctcacatcaaaggtgaagctcaggttaaaggtaccggtttcccggctgacggtccggttatgaccaactctctgaccgctgctgactggtgccgttctaaaaaaacctacccgaacgacaaaaccatcatctctaccttcaaatggtcttacaccaccggtaacggtaaacgttaccgttctaccgctcgtaccacctacaccttcgctaaaccgatggctgctaactacctgaaaaaccagccgatgtacgttttccgtaaaaccgaactgaaacactctaaaaccgaactgaacttcaaagaatggcagaaagctttcaccgacgttatgggtatggacgaactgtacaaaggcggtggcagcggcggtggcagcgctgagggtgacgatcccgcaaaagcggcctttaactccctgcaagcctcagcgaccgaatatatcggttatgcgtgggcgatggttgttgtcattgtcggcgcaactatcggtatcaagctgtttaagaaattcacctcgaaagcaagc

SEQ ID NO: 24 - DNA, 90 bp, Artificial Sequence
  Artificial Sequence
gctgagggtgacgatcccgcaaaagcggcctttaactccctgcaagcctcagcgaccgaatatatcggttatgcgtgggcgatggttgtt

SEQ ID NO: 25 - protein, 30 aa, Artificial Sequence
  Artificial Sequence
AEGDDPAKAAFNSLQASATEYIGYAWAMVV

SEQ ID NO: 26 - protein, 314 aa, Artificial Sequence
  Artificial Sequence
MNNNDLFQTSRQRFLAQLGGLTVAGMLGPSLLTPRRATAAGVSKGEEDNMASLPATHELHIFGSINGVDFDMVGQGTGNPNDGYEELNLKSTKGDLQFSPWILVPHIGYGFHQYLPYPDGMSPFQAAMVDGSGYQVHRTMQFEDGASLTVNYRYTYEGSHIKGEAQVKGTGFPADGPVMTNSLTAADWCRSKKTYPNDKTIISTFKWSYTTGNGKRYRSTARTTYTFAKPMAANYLKNQPMYVFRKTELKHSKTELNFKEWQKAFTDVMGMDELYKGGGSGGGSAEGDDPAKAAFNSLQASATEYIGYAWAMVV

SEQ ID NO: 27 - DNA, 942 bp, Artificial Sequence
  Artificial Sequence
atgaacaataacgatctctttcagacatcacgtcagcgttttttggcacaactcggcggcttaaccgtcgccgggatgctggggccgtcattgttaacgccgcgacgtgcgactgcggcgggcgtttctaaaggtgaagaagacaacatggcttctctgccggctacccacgaactgcacatcttcggttctatcaacggtgttgacttcgacatggttggtcagggtaccggtaacccgaacgacggttacgaagaactgaacctgaaatctaccaaaggtgacctgcagttctctccgtggatcttagttccgcacatcggttacggtttccaccagtacctgccgtacccggacggtatgtctccgttccaggctgctatggttgacggttctggttaccaggttcaccgtaccatgcagttcgaagacggtgcttctctgaccgttaactaccgttacacctacgaaggttctcacatcaaaggtgaagctcaggttaaaggtaccggtttcccggctgacggtccggttatgaccaactctctgaccgctgctgactggtgccgttctaaaaaaacctacccgaacgacaaaaccatcatctctaccttcaaatggtcttacaccaccggtaacggtaaacgttaccgttctaccgctcgtaccacctacaccttcgctaaaccgatggctgctaactacctgaaaaaccagccgatgtacgttttccgtaaaaccgaactgaaacactctaaaaccgaactgaacttcaaagaatggcagaaagctttcaccgacgttatgggtatggacgaactgtacaaaggcggtggcagcggcggtggcagcgctgagggtgacgatcccgcaaaagcggcctttaactccctgcaagcctcagcgaccgaatatatcggttatgcgtgggcgatggttgtt

SEQ ID NO: 28 - protein, 322 aa, Artificial Sequence
  Artificial Sequence
MNNNDLFQTSRQRFLAQLGGLTVAGMLGPSLLTPRRATAADYKDDDDKGVSKGEEDNMASLPATHELHIFGSINGVDFDMVGQGTGNPNDGYEELNLKSTKGDLQFSPWILVPHIGYGFHQYLPYPDGMSPFQAAMVDGSGYQVHRTMQFEDGASLTVNYRYTYEGSHIKGEAQVKGTGFPADGPVMTNSLTAADWCRSKKTYPNDKTIISTFKWSYTTGNGKRYRSTARTTYTFAKPMAANYLKNQPMYVFRKTELKHSKTELNFKEWQKAFTDVMGMDELYKGGGSGGGSAEGDDPAKAAFNSLQASATEYIGYAWAMVV

SEQ ID NO: 29 - DNA, 966 bp, Artificial Sequence
  Artificial Sequence
atgaacaataacgatctctttcagacatcacgtcagcgttttttggcacaactcggcggcttaaccgtcgccgggatgctggggccgtcattgttaacgccgcgacgtgcgactgcggcggattacaaggatgacgatgacaagggcgtttctaaaggtgaagaagacaacatggcttctctgccggctacccacgaactgcacatcttcggttctatcaacggtgttgacttcgacatggttggtcagggtaccggtaacccgaacgacggttacgaagaactgaacctgaaatctaccaaaggtgacctgcagttctctccgtggatcttagttccgcacatcggttacggtttccaccagtacctgccgtacccggacggtatgtctccgttccaggctgctatggttgacggttctggttaccaggttcaccgtaccatgcagttcgaagacggtgcttctctgaccgttaactaccgttacacctacgaaggttctcacatcaaaggtgaagctcaggttaaaggtaccggtttcccggctgacggtccggttatgaccaactctctgaccgctgctgactggtgccgttctaaaaaaacctacccgaacgacaaaaccatcatctctaccttcaaatggtcttacaccaccggtaacggtaaacgttaccgttctaccgctcgtaccacctacaccttcgctaaaccgatggctgctaactacctgaaaaaccagccgatgtacgttttccgtaaaaccgaactgaaacactctaaaaccgaactgaacttcaaagaatggcagaaagctttcaccgacgttatgggtatggacgaactgtacaaaggcggtggcagcggcggtggcagcgctgagggtgacgatcccgcaaaagcggcctttaactccctgcaagcctcagcgaccgaatatatcggttatgcgtgggcgatggttgtt

SEQ ID NO: 30 - DNA, 6 bp, Artificial Sequence
  Artificial Sequence
aggaga

SEQ ID NO: 31 - DNA, 25 bp, Artificial Sequence
  Artificial Sequence
ttaactttaagaaggagatatacat

SEQ ID NO: 32 - protein, 38 aa, Artificial Sequence
  Artificial Sequence
MNNNDLFQASRRRFLAQLGGLTVAGMLGPSLLTPRRAT

SEQ ID NO: 33 - protein, 7 aa, Artificial Sequence
  Artificial Sequence
  MISC_FEATURE (1)..(1): Ser or Thr
  MISC_FEATURE (4)..(4): Any amino acid
XRRXFLK

SEQ ID NO: 34 - protein, 8 aa, Artificial Sequence
  Artificial Sequence
TSRQRFLA

SEQ ID NO: 35 - protein, 38 aa, Artificial Sequence
  Artificial Sequence
MNNNDLFQTSRRRLLAQLGGLTVAGMLGPSLLTPRRAT

SEQ ID NO: 36 - protein, 8 aa, Artificial Sequence
  Artificial Sequence
TSRRRLLA

SEQ ID NO: 37 - protein, 38 aa, Artificial Sequence
  Artificial Sequence
MNNNDIFQASRRRFLAQPGGLTVAGMLGPSLLTPRRAT

SEQ ID NO: 38 - protein, 13 aa, Artificial Sequence
  Artificial Sequence
IFQASRRRFLAQP

SEQ ID NO: 39 - protein, 38 aa, Artificial Sequence
  Artificial Sequence
MNNNELFQASRRRFLAQLGGLTVAGMLGPSLLTPRRAT

SEQ ID NO: 40 - protein, 12 aa, Artificial Sequence
  Artificial Sequence
ELFQASRRRFLA

SEQ ID NO: 41 - protein, 38 aa, Artificial Sequence
  Artificial Sequence
MNNNDLFQTTRRRFLAQLGGLTVAGMLGPSLLTPRRAT

SEQ ID NO: 42 - protein, 8 aa, Artificial Sequence
  Artificial Sequence
TTRRRFLA

SEQ ID NO: 43 - protein, 38 aa, Artificial Sequence
  Artificial Sequence
MNNNDSFQTSRRRFLAQLGGLTVAGMLGPSLLTPRRAT

SEQ ID NO: 44 - protein, 11 aa, Artificial Sequence
  Artificial Sequence
SFQTSRRRFLA

SEQ ID NO: 45 - DNA, 711 bp, Artificial Sequence
  Artificial Sequence
atggtgagcaagggcgaggaggataacatggcctctctcccagcgacacatgagttacacatctttggctccatcaacggtgtggactttgacatggtgggtcagggcaccggcaatccaaatgatggttatgaggagttaaacctgaagtccaccaagggtgacctccagttctccccctggattctggtccctcatatcgggtatggcttccatcagtacctgccctaccctgacgggatgtcgcctttccaggccgccatggtagatggctccggataccaagtccatcgcacaatgcagtttgaagatggtgcctcccttactgttaactaccgctacacctacgagggaagccacatcaaaggagaggcccaggtgaaggggactggtttccctgctgacggtcctgtgatgaccaactcgctgaccgctgcggactggtgcaggtcgaagaagacttaccccaacgacaaaaccatcatcagtacctttaagtggagttacaccactggaaatggcaagcgctaccggagcactgcgcggaccacctacacctttgccaagccaatggcggctaactatctgaagaaccagccgatgtacgtgttccgtaagacggagctcaagcactccaagaccgagctcaacttcaaggagtggcaaaaggcctttaccgatgtgatgggcatggacgagctgtacaagtaa

SEQ ID NO: 46 - protein, 236 aa, Artificial Sequence
  Artificial Sequence
MVSKGEEDNMASLPATHELHIFGSINGVDFDMVGQGTGNPNDGYEELNLKSTKGDLQFSPWILVPHIGYGFHQYLPYPDGMSPFQAAMVDGSGYQVHRTMQFEDGASLTVNYRYTYEGSHIKGEAQVKGTGFPADGPVMTNSLTAADWCRSKKTYPNDKTIISTFKWSYTTGNGKRYRSTARTTYTFAKPMAANYLKNQPMYVFRKTELKHSKTELNFKEWQKAFTDVMGMDELYK

SEQ ID NO: 47 - DNA, 4 bp, Artificial Sequence
  Artificial Sequence
gagg

SEQ ID NO: 48 - DNA, 6 bp, Artificial Sequence
  Artificial Sequence
aggagg

SEQ ID NO: 49 - RNA, 7 nt, Artificial Sequence
  Artificial Sequence
aggaggu

SEQ ID NO: 50 - DNA, 9 bp, Artificial Sequence
  Artificial Sequence
ttaacttta

SEQ ID NO: 51 - DNA, 15 bp, Artificial Sequence
  Artificial Sequence
aaggagacagtcata

SEQ ID NO: 52 - protein, 17 aa, Artificial Sequence
  Artificial Sequence
MSGLNDIFEAQKIEWHE

SEQ ID NO: 53 - protein, 8 aa, Artificial Sequence
  Artificial Sequence
WSHPQFEK

SEQ ID NO: 54 - DNA, 1032 bp, Artificial Sequence
  Artificial Sequence
atgaacaataacgatctctttcagacatcacgtcagcgttttttggcacaactcggcggcttaaccgtcgccgggatgctggggccgtcattgttaacgccgcgacgtgcgactgcggcggattacaaggatgacgatgacaagggcgtttctaaaggtgaagaagacaacatggcttctctgccggctacccacgaactgcacatcttcggttctatcaacggtgttgacttcgacatggttggtcagggtaccggtaacccgaacgacggttacgaagaactgaacctgaaatctaccaaaggtgacctgcagttctctccgtggatcttagttccgcacatcggttacggtttccaccagtacctgccgtacccggacggtatgtctccgttccaggctgctatggttgacggttctggttaccaggttcaccgtaccatgcagttcgaagacggtgcttctctgaccgttaactaccgttacacctacgaaggttctcacatcaaaggtgaagctcaggttaaaggtaccggtttcccggctgacggtccggttatgaccaactctctgaccgctgctgactggtgccgttctaaaaaaacctacccgaacgacaaaaccatcatctctaccttcaaatggtcttacaccaccggtaacggtaaacgttaccgttctaccgctcgtaccacctacaccttcgctaaaccgatggctgctaactacctgaaaaaccagccgatgtacgttttccgtaaaaccgaactgaaacactctaaaaccgaactgaacttcaaagaatggcagaaagctttcaccgacgttatgggtatggacgaactgtacaaaggcggtggcagcggcggtggcagcgctgagggtgacgatcccgcaaaagcggcctttaactccctgcaagcctcagcgaccgaatatatcggttatgcgtgggcgatggttgttgtcattgtcggcgcaactatcggtatcaagctgtttaagaaattcacctcgaaagcaagctgataa

SEQ ID NO: 55 - protein, 342 aa, Artificial Sequence; identical to SEQ ID NO: 22
  Artificial Sequence

SEQ ID NO: 56 - DNA, 819 bp, Artificial Sequence; identical to SEQ ID NO: 17
  Artificial Sequence

SEQ ID NO: 57 - DNA, 1312 bp, Artificial Sequence
  Artificial Sequence
agtgttttagtgtattctttcgcctctttcgttttaggttggtgccttcgtagtggcattacgtattttacccgtttaatggaaacttcctcatgataagctagcaagcaaggagacagtcataatgaacaataacgatctctttcagacatcacgtcagcgttttttggcacaactcggcggcttaaccgtcgccgggatgctggggccgtcattgttaacgccgcgacgtgcgactgcggcggattacaaggatgacgatgacaagggcgtttctaaaggtgaagaagacaacatggcttctctgccggctacccacgaactgcacatcttcggttctatcaacggtgttgacttcgacatggttggtcagggtaccggtaacccgaacgacggttacgaagaactgaacctgaaatctaccaaaggtgacctgcagttctctccgtggatcttagttccgcacatcggttacggtttccaccagtacctgccgtacccggacggtatgtctccgttccaggctgctatggttgacggttctggttaccaggttcaccgtaccatgcagttcgaagacggtgcttctctgaccgttaactaccgttacacctacgaaggttctcacatcaaaggtgaagctcaggttaaaggtaccggtttcccggctgacggtccggttatgaccaactctctgaccgctgctgactggtgccgttctaaaaaaacctacccgaacgacaaaaccatcatctctaccttcaaatggtcttacaccaccggtaacggtaaacgttaccgttctaccgctcgtaccacctacaccttcgctaaaccgatggctgctaactacctgaaaaaccagccgatgtacgttttccgtaaaaccgaactgaaacactctaaaaccgaactgaacttcaaagaatggcagaaagctttcaccgacgttatgggtatggacgaactgtacaaaggcggtggcagcggcggtggcagcgctgagggtgacgatcccgcaaaagcggcctttaactccctgcaagcctcagcgaccgaatatatcggttatgcgtgggcgatggttgttgtcattgtcggcgcaactatcggtatcaagctgtttaagaaattcacctcgaaagcaagctgataagctagcttgaggcatcaataaaacgaaaggctcagtcgaaagactgggcctttcattttatctgttgtttgtcggttaacgcttgtcgtcatcgtccttgtagtcttttttagcagaatctgcggctttcgcatcagcttccggctttgcatcagc

SEQ ID NO: 58 - DNA, 24 bp, Artificial Sequence
  Artificial Sequence
agtgttttagtgtattctttcgcc

SEQ ID NO: 59 - DNA, 16 bp, Artificial Sequence
  Artificial Sequence
gctgatgcaaagccgg

SEQ ID NO: 60 - DNA, 150 bp, Artificial Sequence
  Artificial Sequence
gctgagggtgacgatcccgcaaaagcggcctttaactccctgcaagcctcagcgaccgaatatatcggttatgcgtgggcgatggttgttgtcattataggcgccactatcggtatcaagctgtttaagaaattcacctcgaaagcaagc

SEQ ID NO: 61 - protein, 50 aa, Artificial Sequence
  Artificial Sequence
AEGDDPAKAAFNSLQASATEYIGYAWAMVVVIIGATIGIKLFKKFTSKAS